European Patent Application EP 4 480 499 A1, published December 25, 2024. Title: CONJUGATE OF ANTIBODY-ERIBULIN OR DERIVATIVE THEREOF, INTERMEDIATE THEREOF, PREPARATION METHOD THEREFOR, PHARMACEUTICAL COMPOSITION THEREOF AND USE THEREOF. Applicant: Medilink Therapeutics (SuZhou) Co., Ltd. The sequence listing filed with the application follows.

SEQUENCE LISTING (21 sequences)

SEQ ID NO: 1 - protein, 123 aa, synthetic construct
EGQLVESGGGLVQPGGSLRLSCAASGFTISSYWMNWVRQAPGKGLEWVANIKQDGSEKYYVDSVQGRFTISRDNAKNSLYLQMNSLRAEDTAVYYCARRMYSSGWYWGAFDMWGQGTMVTVSS

SEQ ID NO: 2 - protein, 108 aa, synthetic construct
EIVLTQSPGTLSLSPGERATLSCRASQSVSSIYLAWNQQKPGQAPRLLIYGTFKRATGIPDRFSGSGSGTDFTLTISSLEPEDFAVYYCQQYDTSSITFGQGTRLEIK

SEQ ID NO: 3 - protein, 453 aa, synthetic construct
EGQLVESGGGLVQPGGSLRLSCAASGFTISSYWMNWVRQAPGKGLEWVANIKQDGSEKYYVDSVQGRFTISRDNAKNSLYLQMNSLRAEDTAVYYCARRMYSSGWYWGAFDMWGQGTMVTVSSASTKGPSVFPLAPSSKSTSGGTAALGCLVKDYFPEPVTVSWNSGALTSGVHTFPAVLQSSGLYSLSSVVTVPSSSLGTQTYICNVNHKPSNTKVDKKVEPKSCDKTHTCPPCPAPELLGGPSVFLFPPKPKDTLMISRTPEVTCVVVDVSHEDPEVKFNWYVDGVEVHNAKTKPREEQYNSTYRVVSVLTVLHQDWLNGKEYKCKVSNKALPAPIEKTISKAKGQPREPQVYTLPPSRDELTKNQVSLTCLVKGFYPSDIAVEWESNGQPENNYKTTPPVLDSDGSFFLYSKLTVDKSRWQQGNVFSCSVMHEALHNHYTQKSLSLSPGK

SEQ ID NO: 4 - protein, 215 aa, synthetic construct
EIVLTQSPGTLSLSPGERATLSCRASQSVSSIYLAWNQQKPGQAPRLLIYGTFKRATGIPDRFSGSGSGTDFTLTISSLEPEDFAVYYCQQYDTSSITFGQGTRLEIKRTVAAPSVFIFPPSDEQLKSGTASVVCLLNNFYPREAKVQWKVDNALQSGNSQESVTEQDSKDSTYSLSSTLTLSKADYEKHKVYACEVTHQGLSSPVTKSFNRGEC

SEQ ID NO: 5 - protein, 120 aa, synthetic construct
EVQLLESGGGLVQPGGSLRLSCAASGFTFSSYAMNWVRQAPGKGLEWVSGISGSGGSTYYADSVQGRFTISRDNSKNTLYLQMNSLRAEDTAVYYCAKARSGYDYFFDYWGQGTLVTVSS

SEQ ID NO: 6 - protein, 108 aa, synthetic construct
EIVLTQSPGTLSLSPGERATLSCRASQRISSSFLAWYQQKPGQAPSLLIYGASSRATGIPDRFSGSGSGTDFTLTISSLEPEDFAVFYCQQYSNSPLTFGGGTKVEIK

SEQ ID NO: 7 - protein, 450 aa, synthetic construct
EVQLLESGGGLVQPGGSLRLSCAASGFTFSSYAMNWVRQAPGKGLEWVSGISGSGGSTYYADSVQGRFTISRDNSKNTLYLQMNSLRAEDTAVYYCAKARSGYDYFFDYWGQGTLVTVSSASTKGPSVFPLAPSSKSTSGGTAALGCLVKDYFPEPVTVSWNSGALTSGVHTFPAVLQSSGLYSLSSVVTVPSSSLGTQTYICNVNHKPSNTKVDKKVEPKSCDKTHTCPPCPAPELLGGPSVFLFPPKPKDTLMISRTPEVTCVVVDVSHEDPEVKFNWYVDGVEVHNAKTKPREEQYNSTYRVVSVLTVLHQDWLNGKEYKCKVSNKALPAPIEKTISKAKGQPREPQVYTLPPSRDELTKNQVSLTCLVKGFYPSDIAVEWESNGQPENNYKTTPPVLDSDGSFFLYSKLTVDKSRWQQGNVFSCSVMHEALHNHYTQKSLSLSPGK

SEQ ID NO: 8 - protein, 215 aa, synthetic construct
EIVLTQSPGTLSLSPGERATLSCRASQRISSSFLAWYQQKPGQAPSLLIYGASSRATGIPDRFSGSGSGTDFTLTISSLEPEDFAVFYCQQYSNSPLTFGGGTKVEIKRTVAAPSVFIFPPSDEQLKSGTASVVCLLNNFYPREAKVQWKVDNALQSGNSQESVTEQDSKDSTYSLSSTLTLSKADYEKHKVYACEVTHQGLSSPVTKSFNRGEC

SEQ ID NO: 9 - protein, 5 aa, synthetic construct
SYAMN

SEQ ID NO: 10 - protein, 17 aa, synthetic construct
GISGSGGSTYYADSVQG

SEQ ID NO: 11 - protein, 11 aa, synthetic construct
ARSGYDYFFDY

SEQ ID NO: 12 - protein, 12 aa, synthetic construct
RASQRISSSFLA

SEQ ID NO: 13 - protein, 7 aa, synthetic construct
GASSRAT

SEQ ID NO: 14 - protein, 9 aa, synthetic construct
QQYSNSPLT

SEQ ID NO: 15 - protein, 8 aa, synthetic construct
GFTFSSYA

SEQ ID NO: 16 - protein, 8 aa, synthetic construct
ISGSGGST

SEQ ID NO: 17 - protein, 13 aa, synthetic construct
AKARSGYDYFFDY

SEQ ID NO: 18 - protein, 7 aa, synthetic construct
QRISSSF

SEQ ID NO: 19 - protein, 9 aa, synthetic construct
QQYSNSPLT

SEQ ID NO: 20 - protein, 330 aa, Homo sapiens [sequence omitted]

SEQ ID NO: 21 - protein, 107 aa, Homo sapiens [sequence omitted]